European Patent Specification EP 3 772 539 B1, published June 3, 2026. Title: Sialyltransferases for the production of 6'-sialyllactose. Applicant: Jennewein Biotechnologie GmbH. The sequence listing filed with the application follows.

SEQUENCE LISTING (4 sequences)

SEQ ID NO: 1 - protein, 317 aa, Streptococcus suis
MKRIYICHTVYQVLISLLKMDIKNDTLLSVGIVKNFPNMRNELMAYVNLVEVEEYTFGLRSMIHTLETKNWFSFFKNFEEIIIFLDHRQVGHFLNKHKLPYFLIEDGYNFFKDKRVCHLESIQSSWKRILYRWYFRPATLIGSSPYCQSIEVNDLSLVHPEQAYKPFVEVPRKKLFDSISQERLEAIVQIFGVKSLFNNEVIKERRVLLLTQPLSWEFYVTDEERLEIYLAGLRPYYKDYKIYIKPHPRDSFDYSSLGDGIIIFPQDIPIELFELAGYMNFDVGITYSSSSMDYLDCFDEKVYLHEKFPLPSKTKID

SEQ ID NO: 2 - protein, 322 aa, Streptococcus suis
MRRIYICHTMYQILISLLKMDVERDSLMSVDIIGHFPDVREQLQHVHLIEETERSFDLYSLIARSKTKERLSLLQSYDEVIIFQDHRQVGHFLNKHRIPYSLLEDGYNFFKDKRVCDLESIHSSVWKRLFYQWYFKPTYLIGSSLYCQSIEVNDLSLVQFDEAYKPFVEVPRKQLFDQASPEKVQALLQIFGARAIVADEESSQKRLLLLTQPLSWDYHVTEEELLEIYVAGLAPYREDYTIYIKPHPRDGVDYSFLGKAVVLLPQGIPFELFEMAGSIRFDIGMTYSSSALDFLNCFEEKVYLKDTFPLLSKNDILREGIE

SEQ ID NO: 3 - DNA, 954 bp, Streptococcus suis
atgaaacgcatctacatctgtcacacggtctaccaagttctgattagcctgctgaaaatggatattaaaaatgatacgctgctgtcggttggcattgtcaaaaacttcccgaatatgcgcaacgaactgatggcgtatgtgaatctggtggaagttgaagaatacacctttggtctgcgtagtatgatccacaccctggaaacgaaaaactggttctcctttttcaaaaacttcgaagaaatcatcatttttctggatcatcgccaagtgggccacttcctgaacaaacataaactgccgtattttctgatcgaagatggttacaactttttcaaagacaaacgtgtttgccacctggaaagtattcaaagctcttggaaacgtatcctgtatcgctggtactttcgtccggcaacgctgattggcagttccccgtattgtcagagcatcgaagtcaacgatctgtctctggtgcatccggaacaagcgtacaaaccgttcgtcgaagtgccgcgcaaaaaactgtttgactcaatttcgcaggaacgtctggaagccattgtgcaaatcttcggcgttaaatctctgttcaacaacgaagttatcaaagaacgtcgcgtcctgctgctgacccagccgctgagctgggaattttatgtcacggatgaagaacgcctggaaatttacctggcaggtctgcgtccgtactacaaagactacaaaatttacatcaaaccgcatccgcgcgatagcttcgactattcatcgctgggcgatggtatcattatctttccgcaggacattccgatcgaactgttcgaactggctggctacatgaacttcgatgttggtatcacctatagcagcagcagcatggattacctggactgctttgatgaaaaagtgtatctgcacgaaaaattcccgctgccgtcaaaaaccaaaatcgactaa

SEQ ID NO: 4 - DNA, 969 bp, Streptococcus suis
atgcgtcgtatctatatctgccacaccatgtaccaaattctgatctcgctgctgaaaatggatgttgaacgtgacagtctgatgagcgtggatattatcggccactttccggacgtgcgtgaacagctgcaacatgttcacctgattgaagaaaccgaacgctcgttcgatctgtatagcctgatcgcacgttctaaaacgaaagaacgcctgtccctgctgcagtcatacgatgaagtcattatctttcaggaccatcgtcaagtgggccacttcctgaacaaacatcgcattccgtattcactgctggaagatggttacaactttttcaaagataaacgtgtttgcgacctggaatcgatccatagctctgtctggaaacgcctgttttatcagtggtacttcaaaccgacctatctgattggcagttccctgtactgtcagagtatcgaagttaacgatctgtccctggtccaatttgacgaagcgtataaaccgttcgtcgaagtgccgcgtaaacagctgtttgatcaagcgagcccggaaaaagtccaggccctgctgcaaattttcggtgcgcgtgccatcgttgccgatgaagaatcatcgcagaaacgcctgctgctgctgacccaaccgctgagctgggactatcacgtgacggaagaagaactgctggaaatttatgttgcaggcctggctccgtaccgtgaagattataccatttacatcaaaccgcatccgcgcgatggcgtggactatagctttctgggtaaagcggtggttctgctgccgcagggtattccgtttgaactgttcgaaatggcaggctctattcgctttgatatcggtatgacgtatagctctagtgctctggactttctgaattgcttcgaagaaaaagtttacctgaaagacacgttcccgctgctgagtaaaaatgacatcctgcgtgaaggtattgaataa